European Patent Application EP 4 174 081 A1, published May 3, 2023. Title: NOVEL ATELOCOLLAGEN AND USE THEREOF. Applicant: INTEROLIGO. The sequence listing filed with the application follows.

SEQUENCE LISTING (1 sequence)

SEQ ID NO: 1 - DNA, 30 bp, Artificial Sequence
  GRO aptamer
tggtggtggtggttgtggtggtggtggtgg